European Patent Specification EP 4 135 698 B1, published September 9, 2026. Title: SMALL MOLECULE ANTIVIRAL DRUG TREATMENT FOR HUMAN PAPILLOMAVIRUS INFECTIONS. Applicant: THE TRUSTEES OF INDIANA UNIVERSITY KOVINA THERAPEUTICS, INC. The sequence listing filed with the application follows.

SEQUENCE LISTING (2 sequences)

SEQ ID NO: 1 - protein, 151 aa, Homo sapiens
MFQDPQERPRKLPQLCTELQTTIHDIILECVYCKQQLLRREVYDFAFRDLCIVYRDGNPYAVCDKCLKFYSKISEYRHYCYSLYGTTLEQQYNKPLCDLLIRCINCQKPLCPEEKQRHLDKKQRFHNIRGRWTGRCMSCCRSSRTRRETQL

SEQ ID NO: 2 - protein, 19 aa, Homo sapiens
KEKEEYNSNCSCIACIGLI